European Patent Application EP 4 230 192 A1, published August 23, 2023. Title: Agent for promoting pidermal stem cell increase. Applicant: Shiseido Company, Ltd. The sequence listing filed with the application follows.

SEQUENCE LISTING (12 sequences)

SEQ ID NO: 1 - DNA, 20 bp, Artificial Sequence
  Primer
cacggctctgaccgacatag

SEQ ID NO: 2 - DNA, 19 bp, Artificial Sequence
  Primer
cccagccctctacgacagt

SEQ ID NO: 3 - DNA, 22 bp, Artificial Sequence
  Primer
gtgggatcgagacatgtaagca

SEQ ID NO: 4 - DNA, 19 bp, Artificial Sequence
  Primer
caatccaaatgcggcatct

SEQ ID NO: 5 - DNA, 20 bp, Artificial Sequence
  Primer
gtggcacagaattgctctca

SEQ ID NO: 6 - DNA, 20 bp, Artificial Sequence
  Primer
tcaccctcaaacacctcctc

SEQ ID NO: 7 - DNA, 20 bp, Artificial Sequence
  Primer
ctcgaggtggacaccaccct

SEQ ID NO: 8 - DNA, 20 bp, Artificial Sequence
  Primer
cagctggatggccacatcgc

SEQ ID NO: 9 - DNA, 18 bp, Artificial Sequence
  Primer
tccgggtgagaaaggtga

SEQ ID NO: 10 - DNA, 19 bp, Artificial Sequence
  Primer
gcaggtccagaacctccag

SEQ ID NO: 11 - DNA, 20 bp, Artificial Sequence
  Primer
tgcgcaagttcagcacaatg

SEQ ID NO: 12 - DNA, 20 bp, Artificial Sequence
  Primer
ggcacggtgggatctgaatg